European Patent Application EP 4 410 822 A1, published August 7, 2024. Title: エステル化タンパク質及びその製造方法. Applicant: Ｓｐｉｂｅｒ株式会社. The sequence listing filed with the application follows.

SEQUENCE LISTING (8 sequences)

SEQ ID NO: 1 - protein, 2375 aa, synthetic construct
  REGION 1..2375: note = PRT799
MHHHHHHSSGSSGPGQQGPYGPGASAAAAAGQNGPGSGQQGPGQSGQYGPGQQGPGQQGPGSSAAAAAGPGQYGPGQQGPSASAAAAAGPGSGQQGPGASGQYGPGQQGPGQQGPGSSAAAAAGQYGSGPGQQGPYGSAAAAAGPGSGQYGQGPYGPGASGPGQYGPGQQGPSASAAAAAGSGQQGPGQYGPYASAAAAAGQYGSGPGQQGPYGPGQSGSGQQGPGQQGPYASAAAAAGPGQQGPYGPGSSAAAAAGQYGYGPGQQGPYGPGASGQNGPGSGQYGPGQQGPGQSAAAAAGPGQQGPYGPGASAAAAAGQYGPGQQGPGQYGPGSSGPGQQGPYGPGSSAAAAAGQYGPGQQGPYGPGQSAAAAAGQYQQGPGQQGPYGPGASGPGQQGPYGPGASAAAAAGPGQYGPGQQGPSASAAAAAGQYGSGPGQYGPYGPGQSGPGSGQQGQGPYGPGASAAAAAGQYGPGQQGPYGPGQSAAAAAGPGSGQYGPGASGQNGPGSGQYGPGQQGPGQSAAAAAGQYQQGPGQQGPYGPGASAAAAAGQYGSGPGQQGPYGPGQSGSGQQGPGQQGPYASAAAAAGPGSGQQGPGASGQQGPYGPGASAAAAAGQNGPGSGQQGPGQSGQYGPGQQGPGQQGPGSSAAAAAGPGQYGPGQQGPSASAAAAAGPGSGQQGPGASGQYGPGQQGPGQQGPGSSAAAAAGQYGSGPGQQGPYGSAAAAAGPGSGQYGQGPYGPGASGPGQYGPGQQGPSASAAAAAGSGQQGPGQYGPYASAAAAAGQYGSGPGQQGPYGPGQSGSGQQGPGQQGPYASAAAAAGPGQQGPYGPGSSAAAAAGQYGYGPGQQGPYGPGASGQNGPGSGQYGPGQQGPGQSAAAAAGPGQQGPYGPGASAAAAAGQYGPGQQGPGQYGPGSSGPGQQGPYGPGSSAAAAAGQYGPGQQGPYGPGQSAAAAAGQYQQGPGQQGPYGPGASGPGQQGPYGPGASAAAAAGPGQYGPGQQGPSASAAAAAGQYGSGPGQYGPYGPGQSGPGSGQQGQGPYGPGASAAAAAGQYGPGQQGPYGPGQSAAAAAGPGSGQYGPGASGQNGPGSGQYGPGQQGPGQSAAAAAGQYQQGPGQQGPYGPGASAAAAAGQYGSGPGQQGPYGPGQSGSGQQGPGQQGPYASAAAAAGPGSGQQGPGASGQQGPYGPGASAAAAAGQNGPGSGQQGPGQSGQYGPGQQGPGQQGPGSSAAAAAGPGQYGPGQQGPSASAAAAAGPGSGQQGPGASGQYGPGQQGPGQQGPGSSAAAAAGQYGSGPGQQGPYGSAAAAAGPGSGQYGQGPYGPGASGPGQYGPGQQGPSASAAAAAGSGQQGPGQYGPYASAAAAAGQYGSGPGQQGPYGPGQSGSGQQGPGQQGPYASAAAAAGPGQQGPYGPGSSAAAAAGQYGYGPGQQGPYGPGASGQNGPGSGQYGPGQQGPGQSAAAAAGPGQQGPYGPGASAAAAAGQYGPGQQGPGQYGPGSSGPGQQGPYGPGSSAAAAAGQYGPGQQGPYGPGQSAAAAAGQYQQGPGQQGPYGPGASGPGQQGPYGPGASAAAAAGPGQYGPGQQGPSASAAAAAGQYGSGPGQYGPYGPGQSGPGSGQQGQGPYGPGASAAAAAGQYGPGQQGPYGPGQSAAAAAGPGSGQYGPGASGQNGPGSGQYGPGQQGPGQSAAAAAGQYQQGPGQQGPYGPGASAAAAAGQYGSGPGQQGPYGPGQSGSGQQGPGQQGPYASAAAAAGPGSGQQGPGASGQQGPYGPGASAAAAAGQNGPGSGQQGPGQSGQYGPGQQGPGQQGPGSSAAAAAGPGQYGPGQQGPSASAAAAAGPGSGQQGPGASGQYGPGQQGPGQQGPGSSAAAAAGQYGSGPGQQGPYGSAAAAAGPGSGQYGQGPYGPGASGPGQYGPGQQGPSASAAAAAGSGQQGPGQYGPYASAAAAAGQYGSGPGQQGPYGPGQSGSGQQGPGQQGPYASAAAAAGPGQQGPYGPGSSAAAAAGQYGYGPGQQGPYGPGASGQNGPGSGQYGPGQQGPGQSAAAAAGPGQQGPYGPGASAAAAAGQYGPGQQGPGQYGPGSSGPGQQGPYGPGSSAAAAAGQYGPGQQGPYGPGQSAAAAAGQYQQGPGQQGPYGPGASGPGQQGPYGPGASAAAAAGPGQYGPGQQGPSASAAAAAGQYGSGPGQYGPYGPGQSGPGSGQQGQGPYGPGASAAAAAGQYGPGQQGPYGPGQSAAAAAGPGSGQYGPGASGQNGPGSGQYGPGQQGPGQSAAAAAGQYQQGPGQQGPYGPGASAAAAAGQYGSGPGQQGPYGPGQSGSGQQGPGQQGPYASAAAAAGPGSGQQGSSVDKLAAALEHHHHHH

SEQ ID NO: 2 - protein, 1190 aa, synthetic construct
  REGION 1..1190: note = PRT966
MHHHHHHSSGSSGPGVFGPYGPGASAAAAAGINGPGSGVFGPGISGIYGPGVFGPGVFGPGSSAAAAAGPGIYGPGVFGPSASAAAAAGPGSGVFGPGASGIYGPGVFGPGVFGPGSSAAAAAGIYGSGPGVFGPYGSAAAAAGPGSGIYGIGPYGPGASGPGIYGPGVFGPSASAAAAAGSGVFGPGIYGPYASAAAAAGIYGSGPGVFGPYGPGISGSGVFGPGVFGPYASAAAAAGPGVFGPYGPGSSAAAAAGIYGYGPGVFGPYGPGASGINGPGSGIYGPGVFGPGISAAAAAGPGVFGPYGPGASAAAAAGIYGPGVFGPGIYGPGSSGPGVFGPYGPGSSAAAAAGIYGPGVFGPYGPGISAAAAAGIYVFGPGVFGPYGPGASGPGVFGPYGPGASAAAAAGPGIYGPGVFGPSASAAAAAGIYGSGPGIYGPYGPGISGPGSGVFGIGPYGPGASAAAAAGIYGPGVFGPYGPGISAAAAAGPGSGIYGPGASGINGPGSGIYGPGVFGPGISAAAAAGIYVFGPGVFGPYGPGASAAAAAGIYGSGPGVFGPYGPGISGSGVFGPGVFGPYASAAAAAGPGSGVFGPGASGPGVFGPYGPGASAAAAAGINGPGSGVFGPGISGIYGPGVFGPGVFGPGSSAAAAAGPGIYGPGVFGPSASAAAAAGPGSGVFGPGASGIYGPGVFGPGVFGPGSSAAAAAGIYGSGPGVFGPYGSAAAAAGPGSGIYGIGPYGPGASGPGIYGPGVFGPSASAAAAAGSGVFGPGIYGPYASAAAAAGIYGSGPGVFGPYGPGISGSGVFGPGVFGPYASAAAAAGPGVFGPYGPGSSAAAAAGIYGYGPGVFGPYGPGASGINGPGSGIYGPGVFGPGISAAAAAGPGVFGPYGPGASAAAAAGIYGPGVFGPGIYGPGSSGPGVFGPYGPGSSAAAAAGIYGPGVFGPYGPGISAAAAAGIYVFGPGVFGPYGPGASGPGVFGPYGPGASAAAAAGPGIYGPGVFGPSASAAAAAGIYGSGPGIYGPYGPGISGPGSGVFGIGPYGPGASAAAAAGIYGPGVFGPYGPGISAAAAAGPGSGIYGPGASGINGPGSGIYGPGVFGPGISAAAAAGIYVFGPGVFGPYGPGASAAAAAGIYGSGPGVFGPYGPGISGSGVFGPGVFGPYASAAAAAGPGSGVFGPGAS

SEQ ID NO: 3 - protein, 601 aa, synthetic construct
  REGION 1..601: note = PRT918
MHHHHHHSSGSSGPGVFGPYGPGASAAAAAGINGPGSGVFGPGISGIYGPGVFGPGVFGPGSSAAAAAGPGIYGPGVFGPSASAAAAAGPGSGVFGPGASGIYGPGVFGPGVFGPGSSAAAAAGIYGSGPGVFGPYGSAAAAAGPGSGIYGIGPYGPGASGPGIYGPGVFGPSASAAAAAGSGVFGPGIYGPYASAAAAAGIYGSGPGVFGPYGPGISGSGVFGPGVFGPYASAAAAAGPGVFGPYGPGSSAAAAAGIYGYGPGVFGPYGPGASGINGPGSGIYGPGVFGPGISAAAAAGPGVFGPYGPGASAAAAAGIYGPGVFGPGIYGPGSSGPGVFGPYGPGSSAAAAAGIYGPGVFGPYGPGISAAAAAGIYVFGPGVFGPYGPGASGPGVFGPYGPGASAAAAAGPGIYGPGVFGPSASAAAAAGIYGSGPGIYGPYGPGISGPGSGVFGIGPYGPGASAAAAAGIYGPGVFGPYGPGISAAAAAGPGSGIYGPGASGINGPGSGIYGPGVFGPGISAAAAAGIYVFGPGVFGPYGPGASAAAAAGIYGSGPGVFGPYGPGISGSGVFGPGVFGPYASAAAAAGPGSGVFGPGAS

SEQ ID NO: 4 - protein, 608 aa, synthetic construct
  REGION 1..608: note = PRT313
MHHHHHHSSGSSGPGGQGPYGPGASAAAAAGGNGPGSGQQGPGGSAAAAAGGYGPGGQGPGQQGPGSSAAAAAGPGGYGPGGQGPSASAAAAAGPGSGQQGPGASAAAAAGGYGPGGQGPGQQGPGSSAAAAAGGYGSGPGQQGPYGSAAAAAGPGSGGYGQGPYGPGASAAAAAGPGGYGPGGQGPSASAAAAAGSGQQGPGGYGPYASAAAAAGGYGSGPGQQGPYGPGGSAAAAAGSGQQGPGQQGPYASAAAAAGPGGQGPYGPGSSAAAAAGGYGYGPGGQGPYGPGASAAAAAGGNGPGSGGYGPGQQGPGGSAAAAAGPGGQGPYGPGASAAAAAGGYGPGGQGPGGYGPGSSAAAAAGPGGQGPYGPGSSAAAAAGGYGPGQQGPYGPGGSAAAAAGGYQQGPGGQGPYGPGASAAAAAGPGGQGPYGPGASAAAAAGPGGYGPGGQGPSASAAAAAGGYGSGPGGYGPYGPGGSAAAAAGPGSGQQGQGPYGPGASAAAAAGGYGPGQQGPYGPGGSAAAAAGPGSGGYGPGASAAAAAGGNGPGSGGYGPGQQGPGGSAAAAAGGYQQGPGGQGPYGPGASAAAAAGPGSGQQGPGAS

SEQ ID NO: 5 - protein, 603 aa, synthetic construct
  REGION 1..603: note = PRT1000
MHHHHHHSSGSSCGPGVFGPYGPGASAAAAAGINGPGSGVFGPGISGIYGPGVFGPGVFGPGSSAAAAAGPGIYGPGVFGPSASAAAAAGPGSGVFGPGASGIYGPGVFGPGVFGPGSSAAAAAGIYGSGPGVFGPYGSAAAAAGPGSGIYGIGPYGPGASGPGIYGPGVFGPSASAAAAAGSGVFGPGIYGPYASAAAAAGIYGSGPGVFGPYGPGISGSGVFGPGVFGPYASAAAAAGPGVFGPYGPGSSAAAAAGIYGYGPGVFGPYGPGASGINGPGSGIYGPGVFGPGISAAAAAGPGVFGPYGPGASAAAAAGIYGPGVFGPGIYGPGSSGPGVFGPYGPGSSAAAAAGIYGPGVFGPYGPGISAAAAAGIYVFGPGVFGPYGPGASGPGVFGPYGPGASAAAAAGPGIYGPGVFGPSASAAAAAGIYGSGPGIYGPYGPGISGPGSGVFGIGPYGPGASAAAAAGIYGPGVFGPYGPGISAAAAAGPGSGIYGPGASGINGPGSGIYGPGVFGPGISAAAAAGIYVFGPGVFGPYGPGASAAAAAGIYGSGPGVFGPYGPGISGSGVFGPGVFGPYASAAAAAGPGSGVFGPGASC

SEQ ID NO: 6 - protein, 605 aa, synthetic construct
  REGION 1..605: note = PRT1001
MHHHHHHSSGSSCGPGVFGPYGPGASAAAAAGINGPGSGVFGPGISCGIYGPGVFGPGVFGPGSSAAAAAGPGIYGPGVFGPSASAAAAAGPGSGVFGPGASGIYGPGVFGPGVFGPGSSAAAAAGIYGSGPGVFGPYGSAAAAAGPGSGIYGIGPYGPGASGPGIYGPGVFGPSASAAAAAGSGVFGPGIYGPYASAAAAAGIYGSGPGVFGPYGPGISGSGVFGPGVFGPYASAAAAAGPGVFGPYGPGSSAAAAAGIYGYGPGVFGPYGPGASGINGPGSGIYGPGVFGPGISAAAAAGPGVFGPYGPGASAAAAAGIYGPGVFGPGIYGPGSSGPGVFGPYGPGSSAAAAAGIYGPGVFGPYGPGISAAAAAGIYVFGPGVFGPYGPGASGPGVFGPYGPGASAAAAAGPGIYGPGVFGPSASAAAAAGIYGSGPGIYGPYGPGISGPGSGVFGIGPYGPGASAAAAAGIYGPGVFGPYGPGISAAAAAGPGSGIYGPGASGINGPGSGIYGPGVFGPGISAAAAAGIYVFGPGVFGPYGPGASAAAAAGIYGSGPGVFGPYGPGISGCSGVFGPGVFGPYASAAAAAGPGCSGVFGPGAS

SEQ ID NO: 7 - protein, 1188 aa, synthetic construct
  REGION 1..1188: note = PRT587
MHHHHHHSSGSSGPGQQGPYGPGASAAAAAGQNGPGSGQQGPGQSGQYGPGQQGPGQQGPGSSAAAAAGPGQYGPGQQGPSASAAAAAGPGSGQQGPGASGQYGPGQQGPGQQGPGSSAAAAAGQYGSGPGQQGPYGSAAAAAGPGSGQYGQGPYGPGASGPGQYGPGQQGPSASAAAAAGSGQQGPGQYGPYASAAAAAGQYGSGPGQQGPYGPGQSGSGQQGPGQQGPYASAAAAAGPGQQGPYGPGSSAAAAAGQYGYGPGQQGPYGPGASGQNGPGSGQYGPGQQGPGQSAAAAAGPGQQGPYGPGASAAAAAGQYGPGQQGPGQYGPGSSGPGQQGPYGPGSSAAAAAGQYGPGQQGPYGPGQSAAAAAGQYQQGPGQQGPYGPGASGPGQQGPYGPGASAAAAAGPGQYGPGQQGPSASAAAAAGQYGSGPGQYGPYGPGQSGPGSGQQGQGPYGPGASAAAAAGQYGPGQQGPYGPGQSAAAAAGPGSGQYGPGASGQNGPGSGQYGPGQQGPGQSAAAAAGQYQQGPGQQGPYGPGASAAAAAGQYGSGPGQQGPYGPGQSGSGQQGPGQQGPYASAAAAAGPGSGQQGPGASGQQGPYGPGASAAAAAGQNGPGSGQQGPGQSGQYGPGQQGPGQQGPGSSAAAAAGPGQYGPGQQGPSASAAAAAGPGSGQQGPGASGQYGPGQQGPGQQGPGSSAAAAAGQYGSGPGQQGPYGSAAAAAGPGSGQYGQGPYGPGASGPGQYGPGQQGPSASAAAAAGSGQQGPGQYGPYASAAAAAGQYGSGPGQQGPYGPGQSGSGQQGPGQQGPYASAAAAAGPGQQGPYGPGSSAAAAAGQYGYGPGQQGPYGPGASGQNGPGSGQYGPGQQGPGQSAAAAAGPGQQGPYGPGASAAAAAGQYGPGQQGPGQYGPGSSGPGQQGPYGPGSSAAAAAGQYGPGQQGPYGPGQSAAAAAGQYQQGPGQQGPYGPGASGPGQQGPYGPGASAAAAAGPGQYGPGQQGPSASAAAAAGQYGSGPGQYGPYGPGQSGPGSGQQGQGPYGPGASAAAAAGQYGPGQQGPYGPGQSAAAAAGPGSGQYGPGASGQNGPGSGQYGPGQQGPGQSAAAAAGQYQQGPGQQGPYGPGASAAAAAGQYGSGPGQQGPYGPGQSGSGQQGPGQQGPYASAAAAAGPGSGQQGPGAS

SEQ ID NO: 8 - protein, 12 aa, synthetic construct
  REGION 1..12: note = His6Tag plus Hinge
MHHHHHHSSGSS